European Patent Application EP 4 800 101 A1, published September 2, 2026. Title: Recombinant Attenuated Herpes Simplex Virus Type I Vacccine. Applicant: THE UNIVERSITY OF TOKYO. The sequence listing filed with the application follows.

SEQUENCE LISTING (2 sequences)

SEQ ID NO: 1 - protein, 481 aa, Herpes simplex virus-1
MACRKFCRVYGGQGRRKEEAVPPETKPSRVFPHGPFYTPAEDACLDSPPPETPKPSHTTPPGDAERLCHLQEILAQMYGNQDYPIEDDPSADAADDVDEDAPDDVAYPEEYAEELFLPGDAPGPLIGANDHIPPPCGASPPGIRRRSRDEIGATGFTAEELDAMDREAARAISRGGKPPSTMAKLVTGMGFTIHGALTPGSEGCVFDSSHPDYPQRVIVKAGWYTSTSHEARLLRRLDHPAILPLLDLHVVSGVTCLVLPKYQADLYTYLSRRLNPLGRPQIAAVSRQLLSAVDYIHRQGIIHRDIKTENIFINTPEDICLGDFGAACFVQGSRSSPFPYGIAGTIDTNAPEVLAGDPYTTTVDIWSAGLVIFETAVHNASLFSAPRGPKRGPCDSQITRIIRQAQVHVDEFSPHPESRLTSRYRSRAAGNNRPPYTRPAWTRYYKMDIDVEYLVCKALTFDGALRPSAAELLCLPLFQQK

SEQ ID NO: 2 - protein, 518 aa, Herpes simplex virus-1
MDESRRQRPAGHVAANLSPQGARQRSFKDWLASYIHSNPHGASGRPSGPSLQNAAVSRSSHGCRHRSGLRERLRAGLSRWRMSRSSHRRASPEAPGTAAKLNRPPLRRSQAALTAPPSSPSHILTLTRIRKLCSPVFAINPALHYTTLEIPGARSFGGSGGYGEVQLIREHKLAVKTIKEKEWFAVELIATLLVGECALRAGRTHNIRGFIAPLGFSLQQRQIVFPAYDMDLGKYIGQLASLRTTNPSVSTALHQCFTELARAVVFLNTTCGISHLDIKCANILVMLRSDAVSLRRAVLADFSLVTLNSNSTIARGQFCLQEPDLKSPRMFGMPTALTTANFHTLVGHGYNQPPELLVKYLNNERAEFTNHRLKHDVGLAVDLYALGQTLLELVVSVYVAPSLGVPVTRFPGYQYFNNQLSPDFALALLAYRCVLHPALFVNSAETNTHGLAYDVPEGIRRHLRNPKIRRAFTDRCINYQHTHKAILSSVALPPELKPLLVLVSRLCHTNPCARHALS